European Patent Specification EP 3 423 080 B1, published January 24, 2024. Title: Treatment Method. Applicant: NewSouth Innovations Pty Limited. The sequence listing filed with the application follows.

SEQUENCE LISTING (137 sequences)

SEQ ID NO: 1 - DNA, 1104 bp, Human
atgagctctccgccgcccgcccgcagtggcttttaccgccaggaggtgaccaagacggcctgggaggtgcgcgccgtgtaccgggacctgcagcccgtgggctcgggcgcctacggcgcggtgtgctcggccgtggacggccgcaccggcgctaaggtggccatcaagaagctgtatcggcccttccagtccgagctgttcgccaagcgcgcctaccgcgagctgcgcctgctcaagcacatgcgccacgagaacgtgatcgggctgctggacgtattcactcctgatgagaccctggatgacttcacggacttttacctggtgatgccgttcatgggcaccgacctgggcaagctcatgaaacatgagaagctaggcgaggaccggatccagttcctcgtgtaccagatgctgaaggggctgaggtatatccacgctgccggcatcatccacagagacctgaagcccggcaacctggctgtgaacgaagactgtgagctgaagatcctggacttcggcctggccaggcaggcagacagtgagatgactgggtacgtggtgacccggtggtaccgggctcccgaggtcatcttgaattggatgcgctacacgcagacggtggacatctggtctgtgggctgcatcatggcggagatgatcacaggcaagacgctgttcaagggcagcgaccacctggaccagctgaaggagatcatgaaggtgacggggacgcctccggctgagtttgtgcagcggctgcagagcgatgaggccaagaactacatgaagggcctccccgaattggagaagaaggattttgcctctatcctgaccaatgcaagccctctggctgtgaacctcctggagaagatgctggtgctggacgcggagcagcgggtgacggcaggcgaggcgctggcccatccctacttcgagtccctgcacgacacggaagatgagccccaggtccagaagtatgatgactcctttgacgacgttgaccgcacactggatgaatggaagcgtgttacttacaaagaggtgctcagcttcaagcctccccggcagctgggggccagggtctccaaggagacgcctctgtga

SEQ ID NO: 2 - protein, 367 aa, Human
MSSPPPARSGFYRQEVTKTAWEVRAVYRDLQPVGSGAYGAVCSAVDGRTGAKVAIKKLYRPFQSELFAKRAYRELRLLKHMRHENVIGLLDVFTPDETLDDFTDFYLVMPFMGTDLGKLMKHEKLGEDRIQFLVYQMLKGLRYIHAAGIIHRDLKPGNLAVNEDCELKILDFGLARQADSEMTGYVVTRWYRAPEVILNWMRYTQTVDIWSVGCIMAEMITGKTLFKGSDHLDQLKEIMKVTGTPPAEFVQRLQSDEAKNYMKGLPELEKKDFASILTNASPLAVNLLEKMLVLDAEQRVTAGEALAHPYFESLHDTEDEPQVQKYDDSFDDVDRTLDEWKRVTYKEVLSFKPPRQLGARVSKETPL

SEQ ID NO: 3 - protein, 367 aa, Artificial
  D179A mutant of human P38gamma
MSSPPPARSGFYRQEVTKTAWEVRAVYRDLQPVGSGAYGAVCSAVDGRTGAKVAIKKLYRPFQSELFAKRAYRELRLLKHMRHENVIGLLDVFTPDETLDDFTDFYLVMPFMGTDLGKLMKHEKLGEDRIQFLVYQMLKGLRYIHAAGIIHRDLKPGNLAVNEDCELKILDFGLARQAASEMTGYVVTRWYRAPEVILNWMRYTQTVDIWSVGCIMAEMITGKTLFKGSDHLDQLKEIMKVTGTPPAEFVQRLQSDEAKNYMKGLPELEKKDFASILTNASPLAVNLLEKMLVLDAEQRVTAGEALAHPYFESLHDTEDEPQVQKYDDSFDDVDRTLDEWKRVTYKEVLSFKPPRQLGARVSKETPL

SEQ ID NO: 4 - protein, 441 aa, Human
MAEPRQEFEVMEDHAGTYGLGDRKDQGGYTMHQDQEGDTDAGLKESPLQTPTEDGSEEPGSETSDAKSTPTAEDVTAPLVDEGAPGKQAAAQPHTEIPEGTTAEEAGIGDTPSLEDEAAGHVTQARMVSKSKDGTGSDDKKAKGADGKTKIATPRGAAPPGQKGQANATRIPAKTPPAPKTPPSSGEPPKSGDRSGYSSPGSPGTPGSRSRTPSLPTPPTREPKKVAVVRTPPKSPSSAKSRLQTAPVPMPDLKNVKSKIGSTENLKHQPGGGKVQIINKKLDLSNVQSKCGSKDNIKHVPGGGSVQIVYKPVDLSKVTSKCGSLGNIHHKPGGGQVEVKSEKLDFKDRVQSKIGSLDNITHVPGGGNKKIETHKLTFRENAKAKTDHGAEIVYKSPVVSGDTSPRHLSNVSSTGSIDMVDSPQLATLADEVSASLAKQGL

SEQ ID NO: 5 - protein, 441 aa, Artificial
  Human tau T205E mutant
MAEPRQEFEVMEDHAGTYGLGDRKDQGGYTMHQDQEGDTDAGLKESPLQTPTEDGSEEPGSETSDAKSTPTAEDVTAPLVDEGAPGKQAAAQPHTEIPEGTTAEEAGIGDTPSLEDEAAGHVTQARMVSKSKDGTGSDDKKAKGADGKTKIATPRGAAPPGQKGQANATRIPAKTPPAPKTPPSSGEPPKSGDRSGYSSPGSPGEPGSRSRTPSLPTPPTREPKKVAVVRTPPKSPSSAKSRLQTAPVPMPDLKNVKSKIGSTENLKHQPGGGKVQIINKKLDLSNVQSKCGSKDNIKHVPGGGSVQIVYKPVDLSKVTSKCGSLGNIHHKPGGGQVEVKSEKLDFKDRVQSKIGSLDNITHVPGGGNKKIETHKLTFRENAKAKTDHGAEIVYKSPVVSGDTSPRHLSNVSSTGSIDMVDSPQLATLADEVSASLAKQGL

SEQ ID NO: 6 - DNA, 6581 bp, Artificial
  pAAV-CAG-106-3xHA-p38gamma(MAPK12)-wt
tagctgcgcgctcgctcgctcactgaggccgcccgggcaaagcccgggcgtcgggcgacctttggtcgcccggcctcagtgagcgagcgagcgcgcagagagggagtggccaactccatcactaggggttccttgtagttaatgattaacccgccatgctacttatctacgtagccatgctctaggtaccgggccccccctagaggtagacggtatcttcccatagtaacgccaatagggactttccattgacgtcaatgggtggactatttacggtaaactgcccacttggcagtacatcaagtgtatcatatgccaagtacgccccctattgacgtcaatgacggtaaatggcccgcctggcattatgcccagtacatgaccttatgggactttcctacttggcagtacatctacgtattagtcatcgctattaccatgggtcgaggtgagccccacgttctgcttcactctccccatctcccccccctccccacccccaattttgtatttatttattttttaattattttgtgcagcgatgggggcggggggggggggggcgcgcgccaggcggggcggggcggggcgaggggcggggcggggcgaggcggagaggtgcggcggcagccaatcagagcggcgcgctccgaaagtttccttttatggcgaggcggcggcggcggcggccctataaaaagcgaagcgcgcggcgggcgggagtcgctgcgttgccttcgccccgtgccccgctccgcgccgcctccgcgcccgccgccccggctctgactgaccgcgttactcccacaggtgagcgggcgggacggcccttctcctccgggctgtaattagcgcttggtttaatgacggcttgtttcttttctgtggctgcgtgaaagccttgaggggctccgggagggccctttgtgcggggggagcggctcggggctgtccgcggggggacggctgccttcgggggggacggggcagggcggggttcggcttctggcgtgtgaccggcggctctagagcctctgctaaccatgttcatgccttcttctttttcctacagctcctgggcaacgtgctggttattgtgctgtctcatcattttggcaaagaattggatccactcgagtggagctcgcgactagtcgattcgaattcgatagcttatgtacccatacgatgttccagattacgccatgtacccatacgatgttccagattacgccatgtacccatacgatgttccagattacgccatggggagctctccgccgcccgcccgcagtggcttttaccgccaggaggtgaccaagacggcctgggaggtgcgcgccgtgtaccgggacctgcagcccgtgggctcgggcgcctacggcgcggtgtgctcggccgtggacggccgcaccggcgctaaggtggccatcaagaagctgtatcggcccttccagtccgagctgttcgccaagcgcgcctaccgcgagctgcgcctgctcaagcacatgcgccacgagaacgtgatcgggctgctggacgtattcactcctgatgagaccctggatgacttcacggacttttacctggtgatgccgttcatgggcaccgacctgggcaagctcatgaaacatgagaagctaggcgaggaccggatccagttcctcgtgtaccagatgctgaaggggctgaggtatatccacgctgccggcatcatccacagagacctgaagcccggcaacctggctgtgaacgaagactgtgagctgaagatcctggacttcggcctggccaggcaggcagacagtgagatgactgggtacgtggtgacccggtggtaccgggctcccgaggtcatcttgaattggatgcgctacacgcagacggtggacatctggtctgtgggctgcatcatggcggagatgatcacaggcaagacgctgttcaagggcagcgaccacctggaccagctgaaggagatcatgaaggtgacggggacgcctccggctgagtttgtgcagcggctgcagagcgatgaggccaagaactacatgaagggcctccccgaattggagaagaaggattttgcctctatcctgaccaatgcaagccctctggctgtgaacctcctggagaagatgctggtgctggacgcggagcagcgggtgacggcaggcgaggcgctggcccatccctacttcgagtccctgcacgacacggaagatgagccccaggtccagaagtatgatgactcctttgacgacgttgaccgcacactggatgaatggaagcgtgttacttacaaagaggtgctcagcttcaagcctccccggcagctgggggccagggtctccaaggagacgcctctgtgatctagatcaagcttatcgataatcaacctctggattacaaaatttgtgaaagattgactggtattcttaactatgttgctccttttacgctatgtggatacgctgctttaatgcctttgtatcatgctattgcttcccgtatggctttcattttctcctccttgtataaatcctggttgctgtctctttatgaggagttgtggcccgttgtcaggcaacgtggcgtggtgtgcactgtgtttgctgacgcaacccccactggttggggcattgccaccacctgtcagctcctttccgggactttcgctttccccctccctattgccacggcggaactcatcgccgcctgccttgcccgctgctggacaggggctcggctgttgggcactgacaattccgtggtgttgtcggggaagctgacgtcctttccatggctgctcgcctgtgttgccacctggattctgcgcgggacgtccttctgctacgtcccttcggccctcaatccagcggaccttccttcccgcggcctgctgccggctctgcggcctcttccgcgtcttcgccttcgccctcagacgagtcggatctccctttgggccgcctccccgcatcgataccgtcgactcgctgatcagcctcgactgtgccttctagttgccagccatctgttgtttgcccctcccccgtgccttccttgaccctggaaggtgccactcccactgtcctttcctaataaaatgaggaaattgcatcgcattgtctgagtaggtgtcattctattctggggggtggggtggggcaggacagcaagggggaggattgggaagacaatagcaggcatgctggggatgcggtgggctctatggcttctgaggcggaaagaaccagctggggctcgactagagcatggctacgtagataagtagcatggcgggttaatcattaactacaaggaacccctagtgatggagttggccactccctctctgcgcgctcgctcgctcactgaggccgggcgaccaaaggtcgcccgacgcccgggctttgcccgggcggcctcagtgagcgagcgagcgcgcagagctttttgcaaaagcctaggcctccaaaaaagcctcctcactacttctggaatagctcagaggccgaggcggcctcggcctctgcataaataaaaaaaattagtcagccatggggcggagaatgggcggaactgggcggagttaggggcgggatgggcggagttaggggcgggactatggttgctgactaattgagatgcatgctttgcatacttctgcctgctggggagcctggggactttccacacctggttgctgactaattgagatgcatgctttgcatacttctgcctgctggggagcctggggactttccacaccctaactgacacacattccacagctgcattaatgaatcggccaacgcgcggggagaggcggtttgcgtattgggcgctcttccgcttcctcgctcactgactcgctgcgctcggtcgttcggctgcggcgagcggtatcagctcactcaaaggcggtaatacggttatccacagaatcaggggataacgcaggaaagaacatgtgagcaaaaggccagcaaaaggccaggaaccgtaaaaaggccgcgttgctggcgtttttccataggctccgcccccctgacgagcatcacaaaaatcgacgctcaagtcagaggtggcgaaacccgacaggactataaagataccaggcgtttccccctggaagctccctcgtgcgctctcctgttccgaccctgccgcttaccggatacctgtccgcctttctcccttcgggaagcgtggcgctttctcatagctcacgctgtaggtatctcagttcggtgtaggtcgttcgctccaagctgggctgtgtgcacgaaccccccgttcagcccgaccgctgcgccttatccggtaactatcgtcttgagtccaacccggtaagacacgacttatcgccactggcagcagccactggtaacaggattagcagagcgaggtatgtaggcggtgctacagagttcttgaagtggtggcctaactacggctacactagaagaacagtatttggtatctgcgctctgctgaagccagttaccttcggaaaaagagttggtagctcttgatccggcaaacaaaccaccgctggtagcggtggtttttttgtttgcaagcagcagattacgcgcagaaaaaaaggatctcaagaagatcctttgatcttttctacggggtctgacgctcagtggaacgaaaactcacgttaagggattttggtcatgagattatcaaaaaggatcttcacctagatccttttaaattaaaaatgaagttttaaatcaatctaaagtatatatgagtaaacttggtctgacagttaccaatgcttaatcagtgaggcacctatctcagcgatctgtctatttcgttcatccatagttgcctgactccccgtcgtgtagataactacgatacgggagggcttaccatctggccccagtgctgcaatgataccgcgagacccacgctcaccggctccagatttatcagcaataaaccagccagccggaagggccgagcgcagaagtggtcctgcaactttatccgcctccatccagtctattaattgttgccgggaagctagagtaagtagttcgccagttaatagtttgcgcaacgttgttgccattgctacaggcatcgtggtgtcacgctcgtcgtttggtatggcttcattcagctccggttcccaacgatcaaggcgagttacatgatcccccatgttgtgcaaaaaagcggttagctccttcggtcctccgatcgttgtcagaagtaagttggccgcagtgttatcactcatggttatggcagcactgcataattctcttactgtcatgccatccgtaagatgcttttctgtgactggtgagtactcaaccaagtcattctgagaatagtgtatgcggcgaccgagttgctcttgcccggcgtcaatacgggataataccgcgccacatagcagaactttaaaagtgctcatcattggaaaacgttcttcggggcgaaaactctcaaggatcttaccgctgttgagatccagttcgatgtaacccactcgtgcacccaactgatcttcagcatcttttactttcaccagcgtttctgggtgagcaaaaacaggaaggcaaaatgccgcaaaaaagggaataagggcgacacggaaatgttgaatactcatactcttcctttttcaatattattgaagcatttatcagggttattgtctcatgagcggatacatatttgaatgtatttagaaaaataaacaaataggggttccgcgcacatttccccgaaaagtgccacctgacgtctaagaaaccattattatcatgacattaacctataaaaataggcgtatcacgaggccctttcgtctcgcgcgtttcggtgatgacggtgaaaacctctgacacatgcagctcccggagacggtcacagcttgtctgtaagcggatgccgggagcagacaagcccgtcagggcgcgtcagcgggtgttggcgggtgtcggggctggcttaactatgcggcatcagagcagattgtactgagagtgcaccattcgacgctctcccttatgcgactcctgcattaggaagcagcccagtagtaggttgaggccgttgagcaccgccgccgcaaggaatggtgcatgcaaggagatggcgcccaacagtcccccggccacggggcctgccaccatacccacgccgaaacaagcgctcatgagcccgaagtggcgagcccgatcttccccatcggtgatgtcggcgatataggcgccagcaaccgcacctgtggcgccggtgatgccggccacgatgcgtccggcgtagaggatctggctagcgatgaccctgctgattggttcgctgaccatttccgggtgcgggacggcgttaccagaaactcagaaggttcgtccaaccaaaccgactctgacggcagtttacgagagagatgatagggtctgcttcagtaagccagatgctacacaattaggcttgtacatattgtcgttagaacgcggctacaattaatacataaccttatgtatcatacacatacgatttaggtgacactatagaatacacggaattaattc

SEQ ID NO: 7 - DNA, 6581 bp, Artificial
  pAAV-CAG-106-3xHA-p38gamma(MAPK12)-ca
tagctgcgcgctcgctcgctcactgaggccgcccgggcaaagcccgggcgtcgggcgacctttggtcgcccggcctcagtgagcgagcgagcgcgcagagagggagtggccaactccatcactaggggttccttgtagttaatgattaacccgccatgctacttatctacgtagccatgctctaggtaccgggccccccctagaggtagacggtatcttcccatagtaacgccaatagggactttccattgacgtcaatgggtggactatttacggtaaactgcccacttggcagtacatcaagtgtatcatatgccaagtacgccccctattgacgtcaatgacggtaaatggcccgcctggcattatgcccagtacatgaccttatgggactttcctacttggcagtacatctacgtattagtcatcgctattaccatgggtcgaggtgagccccacgttctgcttcactctccccatctcccccccctccccacccccaattttgtatttatttattttttaattattttgtgcagcgatgggggcggggggggggggggcgcgcgccaggcggggcggggcggggcgaggggcggggcggggcgaggcggagaggtgcggcggcagccaatcagagcggcgcgctccgaaagtttccttttatggcgaggcggcggcggcggcggccctataaaaagcgaagcgcgcggcgggcgggagtcgctgcgttgccttcgccccgtgccccgctccgcgccgcctccgcgcccgccgccccggctctgactgaccgcgttactcccacaggtgagcgggcgggacggcccttctcctccgggctgtaattagcgcttggtttaatgacggcttgtttcttttctgtggctgcgtgaaagccttgaggggctccgggagggccctttgtgcggggggagcggctcggggctgtccgcggggggacggctgccttcgggggggacggggcagggcggggttcggcttctggcgtgtgaccggcggctctagagcctctgctaaccatgttcatgccttcttctttttcctacagctcctgggcaacgtgctggttattgtgctgtctcatcattttggcaaagaattggatccactcgagtggagctcgcgactagtcgattcgaattcgatagcttatgtacccatacgatgttccagattacgccatgtacccatacgatgttccagattacgccatgtacccatacgatgttccagattacgccatggggagctctccgccgcccgcccgcagtggcttttaccgccaggaggtgaccaagacggcctgggaggtgcgcgccgtgtaccgggacctgcagcccgtgggctcgggcgcctacggcgcggtgtgctcggccgtggacggccgcaccggcgctaaggtggccatcaagaagctgtatcggcccttccagtccgagctgttcgccaagcgcgcctaccgcgagctgcgcctgctcaagcacatgcgccacgagaacgtgatcgggctgctggacgtattcactcctgatgagaccctggatgacttcacggacttttacctggtgatgccgttcatgggcaccgacctgggcaagctcatgaaacatgagaagctaggcgaggaccggatccagttcctcgtgtaccagatgctgaaggggctgaggtatatccacgctgccggcatcatccacagagacctgaagcccggcaacctggctgtgaacgaagactgtgagctgaagatcctggacttcggcctggccaggcaggcagccagtgagatgactgggtacgtggtgacccggtggtaccgggctcccgaggtcatcttgaattggatgcgctacacgcagacggtggacatctggtctgtgggctgcatcatggcggagatgatcacaggcaagacgctgttcaagggcagcgaccacctggaccagctgaaggagatcatgaaggtgacggggacgcctccggctgagtttgtgcagcggctgcagagcgatgaggccaagaactacatgaagggcctccccgaattggagaagaaggattttgcctctatcctgaccaatgcaagccctctggctgtgaacctcctggagaagatgctggtgctggacgcggagcagcgggtgacggcaggcgaggcgctggcccatccctacttcgagtccctgcacgacacggaagatgagccccaggtccagaagtatgatgactcctttgacgacgttgaccgcacactggatgaatggaagcgtgttacttacaaagaggtgctcagcttcaagcctccccggcagctgggggccagggtctccaaggagacgcctctgtgatctagatcaagcttatcgataatcaacctctggattacaaaatttgtgaaagattgactggtattcttaactatgttgctccttttacgctatgtggatacgctgctttaatgcctttgtatcatgctattgcttcccgtatggctttcattttctcctccttgtataaatcctggttgctgtctctttatgaggagttgtggcccgttgtcaggcaacgtggcgtggtgtgcactgtgtttgctgacgcaacccccactggttggggcattgccaccacctgtcagctcctttccgggactttcgctttccccctccctattgccacggcggaactcatcgccgcctgccttgcccgctgctggacaggggctcggctgttgggcactgacaattccgtggtgttgtcggggaagctgacgtcctttccatggctgctcgcctgtgttgccacctggattctgcgcgggacgtccttctgctacgtcccttcggccctcaatccagcggaccttccttcccgcggcctgctgccggctctgcggcctcttccgcgtcttcgccttcgccctcagacgagtcggatctccctttgggccgcctccccgcatcgataccgtcgactcgctgatcagcctcgactgtgccttctagttgccagccatctgttgtttgcccctcccccgtgccttccttgaccctggaaggtgccactcccactgtcctttcctaataaaatgaggaaattgcatcgcattgtctgagtaggtgtcattctattctggggggtggggtggggcaggacagcaagggggaggattgggaagacaatagcaggcatgctggggatgcggtgggctctatggcttctgaggcggaaagaaccagctggggctcgactagagcatggctacgtagataagtagcatggcgggttaatcattaactacaaggaacccctagtgatggagttggccactccctctctgcgcgctcgctcgctcactgaggccgggcgaccaaaggtcgcccgacgcccgggctttgcccgggcggcctcagtgagcgagcgagcgcgcagagctttttgcaaaagcctaggcctccaaaaaagcctcctcactacttctggaatagctcagaggccgaggcggcctcggcctctgcataaataaaaaaaattagtcagccatggggcggagaatgggcggaactgggcggagttaggggcgggatgggcggagttaggggcgggactatggttgctgactaattgagatgcatgctttgcatacttctgcctgctggggagcctggggactttccacacctggttgctgactaattgagatgcatgctttgcatacttctgcctgctggggagcctggggactttccacaccctaactgacacacattccacagctgcattaatgaatcggccaacgcgcggggagaggcggtttgcgtattgggcgctcttccgcttcctcgctcactgactcgctgcgctcggtcgttcggctgcggcgagcggtatcagctcactcaaaggcggtaatacggttatccacagaatcaggggataacgcaggaaagaacatgtgagcaaaaggccagcaaaaggccaggaaccgtaaaaaggccgcgttgctggcgtttttccataggctccgcccccctgacgagcatcacaaaaatcgacgctcaagtcagaggtggcgaaacccgacaggactataaagataccaggcgtttccccctggaagctccctcgtgcgctctcctgttccgaccctgccgcttaccggatacctgtccgcctttctcccttcgggaagcgtggcgctttctcatagctcacgctgtaggtatctcagttcggtgtaggtcgttcgctccaagctgggctgtgtgcacgaaccccccgttcagcccgaccgctgcgccttatccggtaactatcgtcttgagtccaacccggtaagacacgacttatcgccactggcagcagccactggtaacaggattagcagagcgaggtatgtaggcggtgctacagagttcttgaagtggtggcctaactacggctacactagaagaacagtatttggtatctgcgctctgctgaagccagttaccttcggaaaaagagttggtagctcttgatccggcaaacaaaccaccgctggtagcggtggtttttttgtttgcaagcagcagattacgcgcagaaaaaaaggatctcaagaagatcctttgatcttttctacggggtctgacgctcagtggaacgaaaactcacgttaagggattttggtcatgagattatcaaaaaggatcttcacctagatccttttaaattaaaaatgaagttttaaatcaatctaaagtatatatgagtaaacttggtctgacagttaccaatgcttaatcagtgaggcacctatctcagcgatctgtctatttcgttcatccatagttgcctgactccccgtcgtgtagataactacgatacgggagggcttaccatctggccccagtgctgcaatgataccgcgagacccacgctcaccggctccagatttatcagcaataaaccagccagccggaagggccgagcgcagaagtggtcctgcaactttatccgcctccatccagtctattaattgttgccgggaagctagagtaagtagttcgccagttaatagtttgcgcaacgttgttgccattgctacaggcatcgtggtgtcacgctcgtcgtttggtatggcttcattcagctccggttcccaacgatcaaggcgagttacatgatcccccatgttgtgcaaaaaagcggttagctccttcggtcctccgatcgttgtcagaagtaagttggccgcagtgttatcactcatggttatggcagcactgcataattctcttactgtcatgccatccgtaagatgcttttctgtgactggtgagtactcaaccaagtcattctgagaatagtgtatgcggcgaccgagttgctcttgcccggcgtcaatacgggataataccgcgccacatagcagaactttaaaagtgctcatcattggaaaacgttcttcggggcgaaaactctcaaggatcttaccgctgttgagatccagttcgatgtaacccactcgtgcacccaactgatcttcagcatcttttactttcaccagcgtttctgggtgagcaaaaacaggaaggcaaaatgccgcaaaaaagggaataagggcgacacggaaatgttgaatactcatactcttcctttttcaatattattgaagcatttatcagggttattgtctcatgagcggatacatatttgaatgtatttagaaaaataaacaaataggggttccgcgcacatttccccgaaaagtgccacctgacgtctaagaaaccattattatcatgacattaacctataaaaataggcgtatcacgaggccctttcgtctcgcgcgtttcggtgatgacggtgaaaacctctgacacatgcagctcccggagacggtcacagcttgtctgtaagcggatgccgggagcagacaagcccgtcagggcgcgtcagcgggtgttggcgggtgtcggggctggcttaactatgcggcatcagagcagattgtactgagagtgcaccattcgacgctctcccttatgcgactcctgcattaggaagcagcccagtagtaggttgaggccgttgagcaccgccgccgcaaggaatggtgcatgcaaggagatggcgcccaacagtcccccggccacggggcctgccaccatacccacgccgaaacaagcgctcatgagcccgaagtggcgagcccgatcttccccatcggtgatgtcggcgatataggcgccagcaaccgcacctgtggcgccggtgatgccggccacgatgcgtccggcgtagaggatctggctagcgatgaccctgctgattggttcgctgaccatttccgggtgcgggacggcgttaccagaaactcagaaggttcgtccaaccaaaccgactctgacggcagtttacgagagagatgatagggtctgcttcagtaagccagatgctacacaattaggcttgtacatattgtcgttagaacgcggctacaattaatacataaccttatgtatcatacacatacgatttaggtgacactatagaatacacggaattaattc

SEQ ID NO: 8 - protein, 4 aa, human
ETPL

SEQ ID NO: 9 - protein, 5 aa, Human
KETPL

SEQ ID NO: 10 - protein, 6 aa, Human
SKETPL

SEQ ID NO: 11 - protein, 7 aa, Human
VSKETPL

SEQ ID NO: 12 - protein, 8 aa, Human
RVSKETPL

SEQ ID NO: 13 - protein, 9 aa, Human
ARVSKETPL

SEQ ID NO: 14 - protein, 10 aa, Human
GARVSKETPL

SEQ ID NO: 15 - protein, 11 aa, Human
LGARVSKETPL

SEQ ID NO: 16 - protein, 12 aa, Human
QLGARVSKETPL

SEQ ID NO: 17 - protein, 13 aa, Human
RQLGARVSKETPL

SEQ ID NO: 18 - protein, 14 aa, Human
PRQLGARVSKETPL

SEQ ID NO: 19 - protein, 15 aa, Human
PPRQLGARVSKETPL

SEQ ID NO: 20 - protein, 16 aa, Human
KPPRQLGARVSKETPL

SEQ ID NO: 21 - protein, 17 aa, Human
FKPPRQLGARVSKETPL

SEQ ID NO: 22 - protein, 18 aa, Human
SFKPPRQLGARVSKETPL

SEQ ID NO: 23 - protein, 19 aa, Human
LSFKPPRQLGARVSKETPL

SEQ ID NO: 24 - protein, 20 aa, Human
VLSFKPPRQLGARVSKETPL

SEQ ID NO: 25 - protein, 21 aa, Human
EVLSFKPPRQLGARVSKETPL

SEQ ID NO: 26 - protein, 23 aa, Human
YKEVLSFKPPRQLGARVSKETPL

SEQ ID NO: 27 - protein, 23 aa, Human
YKEVLSFKPPRQLGARVSKETPL

SEQ ID NO: 28 - protein, 24 aa, Human
TYKEVLSFKPPRQLGARVSKETPL

SEQ ID NO: 29 - protein, 25 aa, Human
VTYKEVLSFKPPRQLGARVSKETPL

SEQ ID NO: 30 - protein, 26 aa, Human
RVTYKEVLSFKPPRQLGARVSKETPL

SEQ ID NO: 31 - protein, 27 aa, Human
KRVTYKEVLSFKPPRQLGARVSKETPL

SEQ ID NO: 32 - protein, 4 aa, Mus musculus
ETAL

SEQ ID NO: 33 - protein, 5 aa, Mus musculus
KETAL

SEQ ID NO: 34 - protein, 6 aa, Mus musculus
PKETAL

SEQ ID NO: 35 - protein, 7 aa, Mus musculus
VPKETAL

SEQ ID NO: 36 - protein, 8 aa, Mus musculus
RVPKETAL

SEQ ID NO: 37 - protein, 9 aa, Mus musculus
ARVPKETAL

SEQ ID NO: 38 - protein, 10 aa, Mus musculus
GARVPKETAL

SEQ ID NO: 39 - protein, 11 aa, Mus musculus
LGARVPKETAL

SEQ ID NO: 40 - protein, 12 aa, Mus musculus
QLGARVPKETAL

SEQ ID NO: 41 - protein, 13 aa, Mus muculus
RQLGARVPKETAL

SEQ ID NO: 42 - protein, 14 aa, Mus musculus
PRQLGARVPKETAL

SEQ ID NO: 43 - protein, 15 aa, Mus musculus
PPRQLGARVPKETAL

SEQ ID NO: 44 - protein, 16 aa, Mus musculus
KPPRQLGARVPKETAL

SEQ ID NO: 45 - protein, 17 aa, Mus musculus
FKPPRQLGARVPKETAL

SEQ ID NO: 46 - protein, 18 aa, Mus musculus
SFKPPRQLGARVPKETAL

SEQ ID NO: 47 - protein, 19 aa, Mus musculus
LSFKPPRQLGARVPKETAL

SEQ ID NO: 48 - protein, 20 aa, Mus musculus
VLSFKPPRQLGARVPKETAL

SEQ ID NO: 49 - protein, 21 aa, Mus musculus
EVLSFKPPRQLGARVPKETAL

SEQ ID NO: 50 - protein, 22 aa, Mus musculus
KEVLSFKPPRQLGARVPKETAL

SEQ ID NO: 51 - protein, 23 aa, Mus musculus
YKEVLSFKPPRQLGARVPKETAL

SEQ ID NO: 52 - protein, 24 aa, Mus musculus
TYKEVLSFKPPRQLGARVPKETAL

SEQ ID NO: 53 - protein, 25 aa, Mus musculus
VTYKEVLSFKPPRQLGARVPKETAL

SEQ ID NO: 54 - protein, 26 aa, Mus musculus
RVTYKEVLSFKPPRQLGARVPKETAL

SEQ ID NO: 55 - protein, 27 aa, Mus musculus
KRVTYKEVLSFKPPRQLGARVPKETAL

SEQ ID NO: 56 - DNA, 20 bp, Mus musculus
gttctgctgcatcttggaca

SEQ ID NO: 57 - DNA, 20 bp, Mus musculus
gaattccgacatgactcagg

SEQ ID NO: 58 - DNA, 27 bp, Mus musculus
gggtgtctccaatgcctgcttcttcag

SEQ ID NO: 59 - DNA, 26 bp, Mus musculus
aagtcacccagcagggaggtgctcag

SEQ ID NO: 60 - DNA, 22 bp, Artificial
  p38alphalox primer
tcctacgagcgtcggcaaggtg

SEQ ID NO: 61 - DNA, 22 bp, Artificial
  p38alphalox reverse primer
agtccccgagagttcctgcctc

SEQ ID NO: 62 - DNA, 30 bp, Artificial
  p38beta forward primer
agaagatgaaggtggaggagtacaagcaag

SEQ ID NO: 63 - DNA, 29 bp, Artificial
  p38beta reverse primer
taacccggatggctgactgttccatttag

SEQ ID NO: 64 - DNA, 21 bp, Artificial
  p38gamma forward primer
tgggctgcgaaggtagaggtg

SEQ ID NO: 65 - DNA, 21 bp, Artificial
  p38gamma reverse primer
gtgtcacgtgctcagggcctg

SEQ ID NO: 66 - DNA, 21 bp, Artificial
  p38delta forward primer
acgtacctgggcgaggcggca

SEQ ID NO: 67 - DNA, 21 bp, Artificial
  p38delta reverse primer
gctcagcttcttgatggccac

SEQ ID NO: 68 - DNA, 20 bp, Artificial
  Wild-type tau forward primer
ctcagcatcccacctgtaac

SEQ ID NO: 69 - DNA, 20 bp, Artificial
  Wild-type tau reverse primer
ccagttgtgtatgtccaccc

SEQ ID NO: 70 - DNA, 19 bp, Artificial
  tau knockout forward primer
aagttcatctgcaccaccg

SEQ ID NO: 71 - DNA, 20 bp, Artificial
  knockout tau reverse primer
tgctcaggtagtggttgtcg

SEQ ID NO: 72 - DNA, 23 bp, Artificial
  Thy1.2-Cre forward primer
gcggtctggcagtaaaaactatc

SEQ ID NO: 73 - DNA, 23 bp, Artificial
  Thy1.2-Cre reverse primer
gtgaaacagcattgctgtcactt

SEQ ID NO: 74 - DNA, 21 bp, Artificial
  Thy1.2-38gammaCA forward primer
aagtcacccagcagggaggtg

SEQ ID NO: 75 - DNA, 22 bp, Artificial
  Thy1.2-38gammaCA reverse primer
tcgtatgggtacatggccaaag

SEQ ID NO: 76 - DNA, 28 bp, Artificial
  tauS46D forward primer
cctgaaagaagatcccctgcagaccccc

SEQ ID NO: 77 - DNA, 18 bp, Artificial
  tauS46D reverse primer
ccagcgtccgtgtcaccc

SEQ ID NO: 78 - DNA, 23 bp, Artificial
  tauT50E forward primer
tcccctgcaggaacccactgagg

SEQ ID NO: 79 - DNA, 18 bp, Artificial
  tauT50E reverse primer
gattctttcaggccagcg

SEQ ID NO: 80 - DNA, 24 bp, Artificial
  tauT52E forward primer
gcagacccccgaagaggacggatc

SEQ ID NO: 81 - DNA, 18 bp, Artificial
  tauT52E reverse primer
aggggagattctttcagg

SEQ ID NO: 82 - DNA, 23 bp, Artificial
  tauT69E forward primer
tgctaagagcgaaccaacagcgg

SEQ ID NO: 83 - DNA, 18 bp, Artificial
  tauT69E reverse primer
tcagaggtttcagagccc

SEQ ID NO: 84 - DNA, 23 bp, Artificial
  tauT71E forward primer
gagcactccagaagcggaagatg

SEQ ID NO: 85 - DNA, 19 bp, Artificial
  tauT71E reverse primer
ttagcatcagaggtttcag

SEQ ID NO: 86 - DNA, 23 bp, Artificial
  tauT111E forward primer
cattggagacgaacccagcctgg

SEQ ID NO: 87 - DNA, 18 bp, Artificial
  tauT111E reverse primer
cctgcttcttcagctgtg

SEQ ID NO: 88 - DNA, 23 bp, Artificial
  tauT153E forward primer
gaagatcgccgaaccgcggggag

SEQ ID NO: 89 - DNA, 18 bp, Artificial
  tauT153E reverse primer
gttttaccatcagccccc

SEQ ID NO: 90 - DNA, 24 bp, Artificial
  tauT181E forward primer
cgctccaaaggaaccacccagctc

SEQ ID NO: 91 - DNA, 18 bp, Artificial
  tauT181E reverse primer
ggcggggtttttgctgga

SEQ ID NO: 92 - DNA, 23 bp, Artificial
  tauS199A forward primer
cggctacagcgcccccggctccc

SEQ ID NO: 93 - DNA, 22 bp, Artificial
  tauS199A reverse primer
ctgcgatcccctgattttggag

SEQ ID NO: 94 - DNA, 23 bp, Artificial
  tauS199D forward primer
cggctacagcgaccccggctccc

SEQ ID NO: 95 - DNA, 22 bp, Artificial
  tauS199D reverse primer
ctgcgatcccctgattttggag

SEQ ID NO: 96 - DNA, 23 bp, Artificial
  tauS202A forward primer
cagccccggcgccccaggcactc

SEQ ID NO: 97 - DNA, 22 bp, Artificial
  tauS202A reverse primer
ctgtagccgctgcgatcccctg

SEQ ID NO: 98 - DNA, 23 bp, Artificial
  tauS202D forward primer
cagccccggcgacccaggcactc

SEQ ID NO: 99 - DNA, 18 bp, Artificial
  tauS202D reverse primer
ctgtagccgctgcgatcc

SEQ ID NO: 100 - DNA, 24 bp, Artificial
  tauS208D forward primer
cactcccggcgaccgctcccgcac

SEQ ID NO: 101 - DNA, 18 bp, Artificial
  tauS208D reverse primer
cctggggagccggggctg

SEQ ID NO: 102 - DNA, 27 bp, Artificial
  tauT212E forward primer
ccgctcccgcgaaccgtcccttccaac

SEQ ID NO: 103 - DNA, 18 bp, Artificial
  tauT212E reverse primer
ctgccgggagtgcctggg

SEQ ID NO: 104 - DNA, 24 bp, Artificial
  tauS235D forward primer
tccacccaaggacccgtcttccgc

SEQ ID NO: 105 - DNA, 18 bp, Artificial
  tauS235D reverse primer
gtacggaccactgccacc

SEQ ID NO: 106 - DNA, 23 bp, Artificial
  tauS404A forward primer
tggggacacggctccacggcatc

SEQ ID NO: 107 - DNA, 24 bp, Artificial
  tauS404A reverse primer
gacaccactggcgacttgtacacg

SEQ ID NO: 108 - DNA, 23 bp, Artificial
  tauS404D forward primer
tggggacacggatccacggcatc

SEQ ID NO: 109 - DNA, 18 bp, Artificial
  tauS404D reverse primer
gacaccactggcgacttg

SEQ ID NO: 110 - DNA, 23 bp, Artificial
  tauT205A forward primer
ctccccaggcgctcccggcagcc

SEQ ID NO: 111 - DNA, 19 bp, Artificial
  tauT205A reverse primer
ccggggctgctgtagccgc

SEQ ID NO: 112 - DNA, 24 bp, Artificial
  tauT205E forward primer
ctccccaggcgaacccggcagccg

SEQ ID NO: 113 - DNA, 18 bp, Artificial
  tauT205E reverse primer
ccggggctgctgtagccg

SEQ ID NO: 114 - DNA, 28 bp, Artificial
  tauS199A T205A forward primer
cccaggcgctcccggcagccgctcccgc

SEQ ID NO: 115 - DNA, 32 bp, Artificial
  tauS199A T205A reverse primer
gagccgggggcgctgtagccgctgcgatcccc

SEQ ID NO: 116 - DNA, 28 bp, Artificial
  tauS199DT205E forward primer
cccaggcgaacccggcagccgctcccgc

SEQ ID NO: 117 - DNA, 32 bp, ARtificial
  tauS199DT205E reverse primer
gagccggggtcgctgtagccgctgcgatcccc

SEQ ID NO: 118 - DNA, 23 bp, Artificial
  tauS396A forward primer
cgtgtacaaggcgccagtggtgt

SEQ ID NO: 119 - DNA, 19 bp, Artificial
  tauS396A reverse primer
atctccgccccgtggtctg

SEQ ID NO: 120 - DNA, 29 bp, Artificial
  tauS396D forward primer
cgtgtacaaggacccagtggtgtctgggg

SEQ ID NO: 121 - DNA, 18 bp, Artificial
  tauS396D reverse primer
atctccgccccgtggtct

SEQ ID NO: 122 - DNA, 31 bp, Artificial
  tauS396AS404A forward primer
tggggacacggctccacggcatctcagcaat

SEQ ID NO: 123 - DNA, 32 bp, Artificial
  tauS396AS404A reverse primer
gacaccactggcgccttgtacacgatctccgc

SEQ ID NO: 124 - DNA, 31 bp, Artificial
  tauS396DS404D forward primer
tggggacacggacccacggcatctcagcaat

SEQ ID NO: 125 - DNA, 32 bp, Artificial
  tauS396DS404D reverse primer
gacaccactgggtccttgtacacgatctccgc

SEQ ID NO: 126 - DNA, 27 bp, Artificial
  tauS422D forward primer
catggtagacgatccccagctcgccac

SEQ ID NO: 127 - DNA, 18 bp, Artificial
  tauS422D reverse primer
tcgatgctgccggtggag

SEQ ID NO: 128 - DNA, 28 bp, Artificial
  tauS199AT205A forward primer
cccaggcgctcccggcagccgctcccgc

SEQ ID NO: 129 - DNA, 32 bp, Artificial; identical to SEQ ID NO: 115
  tauS199AT205A reverse primer

SEQ ID NO: 130 - DNA, 28 bp, Artificial
  tauS199DT205E forward primer
cccaggcgaacccggcagccgctcccgc

SEQ ID NO: 131 - DNA, 32 bp, Artificial; identical to SEQ ID NO: 117
  tauS199DT205E reverse primer

SEQ ID NO: 132 - DNA, 31 bp, Artificial; identical to SEQ ID NO: 122
  tauS396AS404A forward primer

SEQ ID NO: 133 - DNA, 32 bp, Artificial; identical to SEQ ID NO: 123
  tauS396AS404A reverse primer

SEQ ID NO: 134 - DNA, 31 bp, Artificial; identical to SEQ ID NO: 124
  tauS396DS404D forward primer

SEQ ID NO: 135 - DNA, 32 bp, Artificial; identical to SEQ ID NO: 125
  tauS396DS404D reverse primer

SEQ ID NO: 136 - DNA, 47 bp, Artificial
  mCherry PSD-95 forward primer
caagcccagcaatgcctacctgagtgacgtgagcaagggcgaggagg

SEQ ID NO: 137 - DNA, 51 bp, Artificial
  mCherry PSD-95 reverse primer
cgaggttgtgatgtctgggggagcatagctcttgtacagctcgtccatgcc